European Patent Specification EP 3 846 773 B1, published December 20, 2023. Title: Industrial applications of plant cell extracts comprising SOD enzymes of extremophilic micro-organisms. Applicant: Arterra Bioscience Srl. The sequence listing filed with the application follows.

SEQUENCE LISTING (17 sequences)

SEQ ID NO: 1 - DNA, 636 bp, Sulfolobus solfataricus P2
  Gene SOD locus SSO_0316
atgactctccaaattcagtttaaaaagtacgagctacctccattaccctacaagatagatgcattagaaccgtatataagtaaagatataattgatgtacattataacggacatcataaaggctatgtaaatggagcaaattcactcctagaaagactagaaaaagtagtaaaaggagatttacaaacagggcaatatgatattcaaggtattatacgtggtcttacgtttaacattaatggacacaagttacacgccttgtattgggaaaatatggcaccaagtggaaaaggtggtggaaaacctggtggtgcactagcagacttaataaacaagcaatatggtagttttgataggtttaagcaagtatttactgaaactgctaattcactacccgggactggttgggctgttctctattacgatactgagtctggcaatttgcaaattatgacgttcgaaaatcacttccaaaatcatatagcggaaataccaataatattaatactagatgagttcgagcatgcgtactatcttcagtataagaacaagagagctgattacgttaatgcttggtggaatgtagtaaattgggatgcagcggaaaagaagttacagaaatatttaacgaagtaa

SEQ ID NO: 2 - DNA, 645 bp, Aeropyrum pernix K1
  Gene SOD locus APE_0741
atggtgagctttaagaggtacgagctccccccgctaccctacaactacaacgccctggagccctacattatagaggagataatgaagctgcaccaccagaagcatcacaacacgtatgtcaaaggggctaacgccgcactcgagaagatagagaagcatctcaagggcgagatacagatagacgttagggctgtcatgagggacttcagcttcaactacgcaggccacataatgcacaccatattctggcccaacatggccccgcccggcaagggcggtggaacacctggcggcagggtggctgacctcatagagaagcagttcggcggcttcgagaagttcaaggccctcttcagcgccgctgcgaagacggtggagggcgtcgggtggggcgtgctcgcgttcgaccctctgacagaggagctcaggatactgcaggtggagaagcacaacgtcctcatgacggcgggccttgtgcccatactagttattgacgtgtgggagcacgcctactacctccagtacaagaacgacaggggcagctacgtcgagaactggtggaacgtggtcaactgggacgacgttgagaagaggctggagcaggctctaaacaacgcgaagcccctctacctgctcccccagtag

SEQ ID NO: 3 - DNA, 636 bp, Deinococcus radiodurans R1
  Gene SOD locus DR_1279
atggcttacactcttccccaactgccctacgcttacgacgcgcttgagccccatatcgacgcccgcacgatggaaattcaccacaccaagcatcaccagacctacgtggacaacgccaacaaggcgctcgaaggcaccgaattcgccgacctgcccgtcgaacaactcattcagcagctcgaccgcgtgcccgccgacaagaagggcgccctgcgcaacaatgcgggcggccacgccaaccacagcatgttctggcagatcatgggccagggtcagggccagaacggcgccaaccagcccagcggcgaactgctggacgccatcaacagcgccttcggcagcttcgacgccttcaagcagaagttcgaagacgccgccaagacccgcttcggctcgggctgggcgtggctggtcgtcaaggacggcaagctcgatgtcgtgtccaccgccaaccaggacaacccgctgatgggcgaagccatcgcgggcgtcagcggcaccccgattctgggtgtggacgtgtgggaacacgcctactacctcaactaccagaaccgccgccccgactacctcgccgccttctggaacgtggtgaactgggacgaagtctcgaagcgctacgccgccgcgaagtaa

SEQ ID NO: 4 - DNA, 23 bp, Unknown
  Primer forward SsSOD
atgactctccaaattcagtttaa

SEQ ID NO: 5 - DNA, 25 bp, Unknown
  Primer reverse SsSOD
ttacttcgttaaatatttctgtaac

SEQ ID NO: 6 - DNA, 21 bp, Unknown
  Primer forward ApSOD
atggtgagctttaagaggtac

SEQ ID NO: 7 - DNA, 16 bp, Unknown
  Primer reverse ApSOD
ctactgggggagcagg

SEQ ID NO: 8 - DNA, 19 bp, Unknown
  Primer forward DrSOD
atggcttacactcttcccc

SEQ ID NO: 9 - DNA, 15 bp, Unknown
  Primer reverse DrSOD
ttacttcgcggcggc

SEQ ID NO: 10 - DNA, 21 bp, Unknown
  Primer forward SsSOD
gagctacctccattaccctac

SEQ ID NO: 11 - DNA, 20 bp, Unknown
  Primer reverse SsSOD
cttcttttccgctgcatccc

SEQ ID NO: 12 - DNA, 20 bp, Unknown
  Primer forward ApSOD
ctttaagaggtacgagctcc

SEQ ID NO: 13 - DNA, 21 bp, Unknown
  Primer reverse ApSOD
gtgctcccacacgtcaataac

SEQ ID NO: 14 - DNA, 20 bp, Unknown
  Primer forward DrSOD
cttgagccccatatcgacgc

SEQ ID NO: 15 - DNA, 20 bp, Unknown
  Primer reverse DrSOD
cagaaggcggcgaggtagtc

SEQ ID NO: 16 - DNA, 21 bp, Unknown
  Primer forward Cdkn1A
ttcggcccagtggacagcgag

SEQ ID NO: 17 - DNA, 21 bp, Unknown
  Primer reverse Cdkn1A
gcttcctcttggagaagatca